European Patent Application EP 4 806 910 A1, published September 16, 2026. Title: TRI-AGONIST COMPOUND. Applicant: Chengdu Aoda Biotechnology CO.,Ltd. The sequence listing filed with the application follows.

SEQUENCE LISTING (13 sequences)

SEQ ID NO: 1 - protein, 39 aa, synthetic construct
  MOD_RES 2: note = X is Aib
  MOD_RES 13: note = X is alpha MeLeu
  MOD_RES 17: note = X is Lys(2-(2-aminoethoxy) ethoxyacetic acid-gamma Glu-eicosanedioic acid)
  MOD_RES 20: note = X is Aib
YXQGTFTSDYSIXLDKXAQXAFIEYLLEGGPSSGAPPPS

SEQ ID NO: 2 - protein, 38 aa, synthetic construct
  MOD_RES 2: note = X is Aib
  MOD_RES 6: note = X is alpha-MePhe
  MOD_RES 13: note = X is alpha-MeLeu
  MOD_RES 17: note = X is Lys(2-(2-aminoethoxy) ethoxyacetic acid-Gamma Glu-eicosanedioic acid)
  MOD_RES 20: note = X is Aib
  MOD_RES 29: note = X is 5-Ava
YXQGTXTSDYSIXLDKXAQXAFIEYLLEXPSSGAPPPS

SEQ ID NO: 3 - protein, 38 aa, synthetic construct; identical to SEQ ID NO: 2
  MOD_RES 2: note = X is Aib
  MOD_RES 6: note = X is alpha-MePhe
  MOD_RES 13: note = X is alpha-MeLeu
  MOD_RES 17: note = X is Lys(2-(2-aminoethoxy) ethoxyacetic acid-Delta Aad-eicosanedioic acid)
  MOD_RES 20: note = X is Aib
  MOD_RES 29: note = X is 5-Ava

SEQ ID NO: 4 - protein, 38 aa, synthetic construct; identical to SEQ ID NO: 2
  MOD_RES 2: note = X is Aib
  MOD_RES 6: note = X is alpha-MePhe
  MOD_RES 13: note = X is alpha-MeLeu
  MOD_RES 17: note = X is Lys(2-(2-aminoethoxy) ethoxyacetic acid-Epsilon Apm-eicosanedioic acid)
  MOD_RES 20: note = X is Aib
  MOD_RES 29: note = X is 5-Ava

SEQ ID NO: 5 - protein, 38 aa, synthetic construct; identical to SEQ ID NO: 2
  MOD_RES 2: note = X is Aib
  MOD_RES 6: note = X is alpha-MePhe
  MOD_RES 13: note = X is alpha-MeLeu
  MOD_RES 17: note = X is Lys(2-(2-aminoethoxy) ethoxyacetic acid-Zeta Asu-eicosanedioic acid)
  MOD_RES 20: note = X is Aib
  MOD_RES 29: note = X is 5-Ava

SEQ ID NO: 6 - protein, 38 aa, synthetic construct; identical to SEQ ID NO: 2
  MOD_RES 2: note = X is Aib
  MOD_RES 6: note = X is alpha-MePhe(2F)
  MOD_RES 13: note = X is alpha-MeLeu
  MOD_RES 17: note = X is Lys(2-(2-aminoethoxy) ethoxyacetic acid-Gamma Glu-eicosanedioic acid)
  MOD_RES 20: note = X is Aib
  MOD_RES 29: note = X is 5-Ava

SEQ ID NO: 7 - protein, 38 aa, synthetic construct; identical to SEQ ID NO: 2
  MOD_RES 2: note = X is Aib
  MOD_RES 6: note = X is alpha-MePhe(2F)
  MOD_RES 13: note = X is alpha-MeLeu
  MOD_RES 17: note = X is Lys(2-(2-aminoethoxy) ethoxyacetic acid-Delta Aad-eicosanedioic acid)
  MOD_RES 20: note = X is Aib
  MOD_RES 29: note = X is 5-Ava

SEQ ID NO: 8 - protein, 38 aa, synthetic construct; identical to SEQ ID NO: 2
  MOD_RES 2: note = X is Aib
  MOD_RES 6: note = X is alpha-MePhe(2F)
  MOD_RES 13: note = X is alpha-MePhe(2F)
  MOD_RES 17: note = X is Lys(2-(2-aminoethoxy) ethoxyacetic acid-Epsilon Apm-eicosanedioic acid)
  MOD_RES 20: note = Aib
  MOD_RES 29: note = X is 5-Ava

SEQ ID NO: 9 - protein, 38 aa, synthetic construct; identical to SEQ ID NO: 2
  MOD_RES 2: note = X is Aib
  MOD_RES 6: note = X is alpha-MePhe(2F)
  MOD_RES 13: note = X is alpha-MeLeu
  MOD_RES 17: note = X is Lys(2-(2-aminoethoxy) ethoxyacetic acid-Zeta Asu-eicosanedioic acid)
  MOD_RES 20: note = X is Aib
  MOD_RES 29: note = X is 5-Ava

SEQ ID NO: 10 - protein, 38 aa, synthetic construct; identical to SEQ ID NO: 2
  MOD_RES 2: note = X is Aib
  MOD_RES 6: note = X is alpha-MePhe
  MOD_RES 13: note = X is alpha-MeLeu
  MOD_RES 17: note = X is Lys(2-(2-aminoethoxy) ethoxyacetic acid-2-(2-aminoethoxy) ethoxyacetic acid-Gamma Glu-eicosanedioic acid)
  MOD_RES 20: note = X is Aib
  MOD_RES 29: note = X is 5-Ava

SEQ ID NO: 11 - protein, 38 aa, synthetic construct; identical to SEQ ID NO: 2
  MOD_RES 2: note = X is Aib
  MOD_RES 6: note = X is alpha-MePhe
  MOD_RES 13: note = X is alpha-MeLeu
  MOD_RES 17: note = X is Lys(COCH2PEG5-Gamma Glu-eicosanedioic acid)
  MOD_RES 20: note = X is Aib
  MOD_RES 29: note = X is 5-Ava

SEQ ID NO: 12 - protein, 38 aa, synthetic construct; identical to SEQ ID NO: 2
  MOD_RES 2: note = X is Aib
  MOD_RES 6: note = X is alpha-MePhe(2F)
  MOD_RES 13: note = X is alpha-MeLeu
  MOD_RES 17: note = X is Lys(2-(2-aminoethoxy) ethoxyacetic acid-2-(2-aminoethoxy) ethoxyacetic acid-Gamma Glu-eicosanedioic acid)
  MOD_RES 20: note = X is Aib
  MOD_RES 29: note = X is 5-Ava

SEQ ID NO: 13 - protein, 38 aa, synthetic construct; identical to SEQ ID NO: 2
  MOD_RES 2: note = X is Aib
  MOD_RES 6: note = X is alpha-MePhe(2F)
  MOD_RES 13: note = X is alpha-MeLeu
  MOD_RES 17: note = X is Lys(COCH2PEG5-Gamma Glu-eicosanedioic acid)
  MOD_RES 20: note = X is Aib
  MOD_RES 29: note = X is 5-Ava